European Patent Specification EP 3 919 505 B1, published August 30, 2023. Title: CAS9-NUCLEIC ACID COMPLEXES AND USES RELATED THERETO. Applicant: Emory University. The sequence listing filed with the application follows.

SEQUENCE LISTING (45 sequences)

SEQ ID NO: 1 - protein, 1628 aa, Artificial Sequence
  synthetic construct
MNFKILPIAIDLGVKNTGVFSAFYQKGTSLERLDNKNGKVYELSKDSYTLLMNNRTARRHQRRGIDRKQLVKRLFKLIWTEQLNLEWDKDTQQAISFLFNRRGFSFITDGYSPEYLNIVPEQVKAILMDIFDDYNGEDDLDSYLKLATEQESKISEIYNKLMQKILEFKLMKLCTDIKDDKVSTKTLKEITSYEFELLADYLANYSESLKTQKFSYTDKQGNLKELSYYHHDKYNIQEFLKRHATINDRILDTLLTDDLDIWNFNFEKFDFDKNEEKLQNQEDKDHIQAHLHHFVFAVNKIKSEMASGGRHRSQYFQEITNVLDENNHQEGYLKNFCENLHNKKYSNLSVKNLVNLIGNLSNLELKPLRKYFNDKIHAKADHWDEQKFTETYCHWILGEWRVGVKDQDKKDGAKYSYKDLCNELKQKVTKAGLVDFLLELDPCRTIPPYLDNNNRKPPKCQSLILNPKFLDNQYPNWQQYLQELKKLQSIQNYLDSFETDLKVLKSSKDQPYFVEYKSSNQQIASGQRDYKDLDARILQFIFDRVKASDELLLNEIYFQAKKLKQKASSELEKLESSKKLDEVIANSQLSQILKSQHTNGIFEQGTFLHLVCKYYKQRQRARDSRLYIMPEYRYDKKLHKYNNTGRFDDDNQLLTYCNHKPRQKRYQLLNDLAGVLQVSPNFLKDKIGSDDDLFISKWVEHIRGFKKACEDSLKIQKDNRGLLNHKINIARNTKGKCEKEIFNLICKIEGSEDKKGNYKHGLAYELGVLLFGEPNEASKPEFDRKIKKFNSIYSFAQIQQIAFAERKGNANTCAVCSADNAHRMQQIKITEPVEDNKDKIILSAKAQRLPAIPTRIVDGAVKKMATILAKNIVDDNWQNIKQVLSAKHQLHIPIITESNAFEFEPALADVKGKSLKDRRKKALERISPENIFKDKNNRIKEFAKGISAYSGANLTDGDFDGAKEELDHIIPRSHKKYGTLNDEANLICVTRGDNKNKGNRIFCLRDLADNYKLKQFETTDDLEIEKKIADTIWDANKKDFKFGNYRSFINLTPQEQKAFRHALFLADENPIKQAVIRAINNRNRTFVNGTQRYFAEVLANNIYLRAKKENLNTDKISFDYFGIPTIGNGRGIAEIRQLYEKVDSDIQAYAKGDKPQASYSHLIDAMLAFCIAADEHRNDGSIGLEIDKNYSLYPLDKNTGEVFTKDIFSQIKITDNEFSDKKLVRKKAIEGFNTHRQMTRDGIYAENYLPILIHKELNEVRKGYTWKNSEEIKIFKGKKYDIQQLNNLVYCLKFVDKPISIDIQISTLEELRNILTTNNIAATAEYYYINLKTQKLHEYYIENYNTALGYKKYSKEMEFLRSLAYRSERVKIKSIDDVKQVLDKDSNFIIGKITLPFKKEWQRLYREWQNTTIKDDYEFLKSFFNVKSITKLHKKVRKDFSLPISTNEGKFLVKRKTWDNNFIYQILNDSDSRADGTKPFIPAFDISKNEIVEAIIDSFTSKNIFWLPKNIELQKVDNKNIFAIDTSKWFEVETPSDLRDIGIATIQYKIDNNSRPKVRVKLDYVIDDDSKINYFMNHSLLKSRYPDKVLEILKQSTIIEFESSGFNKTIKEMLGMKLAGIYNETSNN

SEQ ID NO: 2 - DNA, 4889 bp, Artificial Sequence
  synthetic construct
atgaatttcaaaatattgccaatagcaatagatttaggtgttaaaaatactggtgtctttagcgcattttatcaaaaaggaacttctcttgagagattggataataaaaatggcaaagtatatgaactatcaaaagattcttatactttattgatgaataatagaacagcaagaagacatcaaagaagagggatagatagaaagcagctagtcaaaaggctctttaagcttatttggacagagcagctaaatttagagtgggataaagacactcaacaagcaattagctttttatttaatcgtagaggttttagttttattactgatggttattcgcctgaatatttaaatattgttccagagcaagtaaaagcgatacttatggatatatttgatgattacaacggtgaagatgatttagacagttatttaaaattagctactgagcaagaaagcaaaatttctgaaatttataacaagctaatgcaaaaaatattagagtttaaattaatgaaattatgtactgatattaaggatgataaagtaagtactaaaacgcttaaagaaatcacaagctatgaatttgagttattagctgattatttagcaaactatagcgagagtttaaaaacacaaaaatttagttatacagataaacaaggtaatttaaaagagctaagctactatcatcatgataaatataatattcaagaatttctaaagcgacatgctactataaatgatcgaattttagatactcttttaactgatgatttagatatttggaattttaattttgagaaatttgattttgataagaatgaagaaaagcttcagaatcaggaagataaagatcatatacaagcgcatttacatcattttgtttttgcagtaaataaaataaaaagtgaaatggcaagtggtggtcgtcatcgtagccaatattttcaagagataacaaatgtgctagatgaaaataatcatcaagagggatatctcaagaatttctgtgaaaatttgcataataaaaaatattcaaatttaagtgttaaaaatttagttaatctaattggtaacctaagtaatttagagctaaaaccgctaagaaaatattttaatgacaaaattcacgcaaaagctgatcattgggatgagcaaaagtttacagaaacttattgccactggatattaggagagtggcgagtaggtgtcaaagatcaagataagaaagatggcgctaaatatagttataaagatctgtgtaatgaattaaaacaaaaagttactaaggctggtttggtagattttttattagagttagatccatgtagaactataccaccatatctggataacaataaccgtaaaccaccaaaatgtcaaagtttgattttaaatccgaagtttttagataatcaatatccaaactggcaacaatatttacaagaattaaagaaactacaaagtattcaaaattatttagacagttttgaaactgatttaaaagtcttaaagtcaagtaaagatcaaccatattttgttgaatacaagagttcaaatcagcaaatagcaagtggtcaaagagattataaagatttagatgctcgaatattacagtttatatttgatagggtaaaagctagtgatgagttgcttttgaatgagatttattttcaggctaaaaaacttaaacaaaaagctagctctgagttagaaaaactcgagtcgagcaaaaagctagatgaagttatagcaaatagtcaactatcacagatactaaagtctcaacatacaaatggtatttttgaacagggtacttttttgcatttggtttgtaaatattataaacaaagacaaagagcgagagactctaggctatatattatgcctgaatatcgttatgataaaaaactacataaatataacaatacaggcaggtttgatgatgataatcagctgctaacatattgtaatcataagccaagacaaaaaagataccaattgttaaatgatttagctggggtgttgcaggtatcacctaattttttgaaagataaaattggttctgatgatgatctatttattagcaaatggttggtagagcatattagaggatttaaaaaagcttgtgaagatagtttaaaaatacaaaaagacaatagaggattattaaatcataaaataaatatagctaggaatacaaaaggcaaatgtgaaaaagaaatatttaatttaatatgtaaaatagaaggttcagaagataaaaaaggtaattacaagcatggtttagcttacgaattaggagtacttttatttggtgaacctaatgaagctagtaaacctgagttcgatagaaaaattaaaaaatttaactcaatatacagttttgcacagattcaacaaattgcttttgcagagcgtaaaggcaatgctaacacttgtgcagtttgtagtgctgataatgctcatagaatgcaacaaattaagatcactgagcctgtagaggacaataaagatagataatcttaagtgccaaagctcagagactaccagcgattccaactagaatagttgacggtgcggttaagaaaatggcaactatattagctaaaaatatagttgatgataattggcagaatatcaaacaagttttatcagcaaaacatcagttacatatacctattatcacagaatcaaatgcttttgagtttgaaccagcattagctgatgtaaaaggtaagagcctaaaagataggagaaaaaaagcattagagagaataagtcctgaaaatatattcaaggataaaaacaatagaataaaagaatttgctaaaggtatatcagcatatagtggtgctaatttaactgatggcgattttgatggtgcaaaagaagaattagatcatataatacctcgttcacataaaaaatacggtactctaaatgatgaagcaaatctaatttgtgtaactcgtggtgataataaaaataaaggtaatagaattttctgcctacgtgatcttgcagataactataaactaaaacagtttgagacaactgatgatttagaaattgaaaagaagatagctgatacaatctgggatgctaacaagaaagattttaaatttggtaattatcgtagttttattaacctaacaccacaagagcagaaagcatttcgtcacgcgctatttctggctgatgaaaatcctatcaaacaagcagtcataagagcgataaataatcgtaatcgtacatttgtaaatggcactcaacgctattttgcagaagtactggcaaacaatatctatctaagggctaaaaaagaaaatctaaatacagataaaatttcatttgattattttggtattccaactataggtaatggtagaggtattgctgaaatccgtcaactttatgaaaaagttgatagtgatatacaagcttatgcaaaaggtgataaacctcaagctagctactctcacctaatagatgcgatgctggctttttgtattgctgctgatgaacacagaaatgatggaagtataggtctagaaatcgataaaaattatagtttatatccattagataaaaatacaggagaagtctttaccaaagatatttttagtcaaattaaaattactgataatgagtttagcgataaaaaattagtaagaaaaaaagctatagagggctttaacacgcatagacaaatgactagagatggcatttatgcagaaaattacctaccaatactaatccataaagaactaaatgaagttagaaaaggctatacttggaaaaatagtgaagaaataaaaatattcaaaggtaaaaagtacgatatacaacaattgaataaccttgtgtattgtctaaaatttgtagataaacctatatctatagatatacaaattagtaccttagaagagttaagaaatatattaacaacaaataatatagctgctacagcagaatactattatataaatctaaaaacccaaaaattacatgagtattatatcgaaaactataatactgccttaggttataaaaaatacagtaaagaaatggagtttttgagaagcttagcttatcgtagcgaaagggtaaaaattaaatcaatagatgatgtaaagcaggttttggataaggatagtaactttatcatcggtaagattactttaccatttaaaaaagagtggcaaagactatatcgtgagtggcaaaatacaactatcaaagatgattatgagtttttaaaatcattctttaatgttaaaagtattactaagttgcataaaaaagttagaaaagatttctctttacctatttctacaaatgaaggtaaattcctggtcaaaagaaaaacatgggataacaattttatctatcagatattaaatgattctgattctagagcagacggaacaaagccatttattccagcttttgacatttctaaaaatgaaatagtcgaagccataattgattcatttacatcaaaaaatattttttggctgcctaaaaatatagaattacaaaaggtggataataaaaacatttttgctatagatactagtaaatggttcgaagtagaaacacctagtgatcttagagacattggaatagcaacaattcaatacaagatagataataattctcgccctaaagtcagagttaaacttgattatgttatcgatgatgatagtaagataaattattttatgaatcattctttattaaaatcaagatatcctgacaaagttttagaaattttaaaacaatcaactattatagaatttgaaagttcaggttttaataaaactatcaaagaaatgcttggtatgaaattagcaggtatttataatgaaacatctaataattag

SEQ ID NO: 3 - RNA, 78 nt, Artificial Sequence
  Synthetic construct
  misc_feature (6)..(6): where n is any nucleotide.
  misc_feature (45)..(46): where n is any nucleotide.
guugunuagauuauuugguauguacuuguguuaguuuaaaguagnncuagaaaauucacuuuuagaccuacuuauuuu

SEQ ID NO: 4 - RNA, 111 nt, Artificial Sequence
  synthetic construct
guaccaaauaauuaaugcucuguaaucauuuaaaaguauuuugaacggaccucuguuugacacgucugaauaacuaaaaagcaaaaauuugccaccuaaguggcuuuuuuu

SEQ ID NO: 5 - RNA, 13 nt, Artificial Sequence
  Synthetic construct
guaccaaauaauu

SEQ ID NO: 6 - protein, 21 aa, Artificial Sequence
  Synthetic construct
MNNRTARRHQRRGIDRKQLVK

SEQ ID NO: 7 - protein, 35 aa, Artificial Sequence
  Synthetic construct
KNIVDDNWQNIKQVLSAKHQLHIPIITESNAFEFE

SEQ ID NO: 8 - protein, 31 aa, Artificial Sequence
  Synthetic construct
AKGDKPQASYSHLIDAMLAFCIAADEHRNDG

SEQ ID NO: 9 - DNA, 4887 bp, Homo sapiens
atgaactttaagatcctccctattgccatcgacctgggcgtgaagaacaccggcgtgtttagcgccttttaccagaagggcaccagcctggagagactggataataagaacggcaaggtgtatgagctcagcaaggacagctataccctgctcatgaataacaggaccgctagaaggcaccaaagaagaggcatcgacagaaagcagctggtcaagagactgttcaaactgatttggacagagcaactgaacctggagtgggataaggacacccagcaggctatctccttcctcttcaacaggagaggcttcagcttcattaccgacggctactcccctgagtatctgaacattgtccccgaacaggtcaaggccatcctgatggacatctttgacgactacaacggagaggatgatctcgactcctatctgaagctggctaccgaacaggaaagcaagatttccgagatctacaacaagctcatgcaaaagattctggaattcaagctcatgaagctgtgtaccgatatcaaggacgacaaggtcagcaccaaaaccctcaaagaaatcaccagctatgaatttgagctgctggccgattacctggctaattacagcgagagcctgaagacccagaagttcagctataccgataagcaaggcaatctcaaggagctgagctactatcaccatgacaagtacaatattcaggagtttctgaagaggcatgctaccatcaatgataggatcctcgacacactgctcaccgatgacctggatatctggaactttaactttgagaaattcgactttgataagaatgaagaaaagctgcaaaatcaggaagacaaggatcacattcaggctcacctgcaccacttcgtcttcgccgtcaacaagatcaagagcgaaatggcttccggaggcaggcacaggagccagtacttccaggaaatcaccaacgtcctggacgagaacaaccaccaggaaggctacctcaagaatttctgtgagaacctgcacaacaagaaatatagcaacctgtccgtgaaaaacctcgtcaacctcatcggcaacctgagcaatctggagctgaagcccctgaggaagtacttcaacgacaagattcatgccaaggctgaccactgggacgagcagaagttcacagagacatactgtcactggatcctgggagaatggagggtgggcgtcaaagaccaggacaaaaaagatggagctaagtacagctacaaagatctgtgtaatgagctcaaacagaaggtgacaaaagccggactggtggacttcctgctggagctggatccctgcaggacaattcccccctatctcgacaacaataacaggaagcctcccaagtgccaaagcctcatcctcaaccccaagttcctcgacaatcagtatcccaattggcagcagtacctgcaagaactgaaaaaactgcaaagcattcaaaactacctcgattccttcgagaccgacctcaaagtcctcaaaagcagcaaggaccaaccctacttcgtcgaatacaagagcagcaaccagcagatcgcctccggacagagagactacaaagacctcgacgccaggattctgcaattcatcttcgacagagtcaaggcttccgacgaactgctgctgaatgaaatctattttcaagctaaaaagctcaagcagaaagccagcagcgaactcgaaaaactggagtcctccaagaaactcgacgaggtgattgccaatagccaactcagccagatcctgaagagccagcatacaaatggcatcttcgagcaaggcacatttctgcatctggtgtgtaaatactacaaacaaagacagagggctagggacagcagactctatatcatgcccgagtacagatacgataaaaaactgcataaatacaacaacaccggcaggtttgacgacgataaccaactgctcacctactgcaaccacaagcctaggcaaaaaaggtatcagctgctgaacgacctggctggagtgctccaagtctcccctaatttcctcaaggataaaattggatccgacgatgacctcttcatctccaagtggctggtcgagcacatcagaggcttcaagaaggcctgcgaagattccctgaaaatccagaaggacaacaggggactcctgaatcataagattaatatcgctagaaataccaagggcaaatgcgagaaggagatcttcaacctgatctgcaaaatcgaaggctccgaggataagaaaggcaactataagcatggcctggcttatgagctcggagtgctcctgttcggagagcccaatgaggcctccaagcctgaatttgacaggaagatcaagaagtttaatagcatctactccttcgcccagatccaacaaatcgccttcgctgaaaggaagggcaacgctaacacctgcgccgtgtgcagcgctgataatgctcacaggatgcagcagatcaagatcacagaacccgtggaagacaataaagacaagatcatcctcagcgctaaggctcagagactgcccgctattcctacaagaatcgtggacggagccgtcaagaaaatggccaccatcctggccaaaaacatcgtggatgataattggcaaaatattaaacaggtcctgtccgccaagcaccagctccacattcccatcatcaccgagtccaatgctttcgagttcgaacccgccctggctgacgtgaaaggcaaatccctcaaggacagaagaaagaaggccctggagagaatttcccctgagaacatctttaaggacaaaaataacagaattaaagagtttgctaagggaatttccgcctacagcggcgccaatctgacagatggcgacttcgatggcgctaaagaagagctcgaccacatcattcccagaagccacaagaagtatggaaccctcaacgatgaggccaacctcatctgcgtcaccaggggcgacaataaaaataaaggcaataggatcttctgtctgagagacctggccgataactacaaactgaaacagttcgaaaccaccgacgacctggagattgagaagaaaatcgccgacaccatctgggacgctaataaaaaagactttaagttcggaaactacaggagcttcattaacctgacaccccaggaacagaaagcctttaggcatgccctctttctggccgatgagaaccctatcaagcaagccgtcatcagggccatcaacaacaggaataggaccttcgtcaatggcacccagaggtactttgccgaggtgctggccaataacatctatctcagggctaaaaaggagaatctcaatacagacaaaatctcctttgactattttggaatccctaccatcggaaatggcaggggaatcgctgagattagacagctgtacgagaaagtcgacagcgatatccaagcctacgccaagggagataagcctcaggcttcctatagccacctcatcgacgctatgctggccttttgcatcgccgccgacgagcacagaaatgatggctccatcggactggaaatcgacaagaattacagcctctaccccctcgacaaaaacacaggagaggtgttcacaaaagatattttcagccagattaagattacagacaacgaatttagcgataagaaactggtgagaaagaaagctatcgagggatttaatacccataggcaaatgaccagggacggcatttacgctgagaactatctccccatcctcatccacaaggaactgaacgaagtcagaaaaggatatacctggaaaaatagcgaggaaattaagattttcaaaggaaaaaagtatgacatccagcagctcaacaacctcgtgtattgcctcaagttcgtggacaagcccatttccatcgacatccagatcagcacactggaagagctgaggaatatcctgaccacaaataacattgccgctaccgctgagtattattacattaatctcaaaacacagaaactgcatgaatattacatcgagaactacaataccgccctgggctataagaagtattccaaggaaatggagttcctcaggtccctcgcctataggagcgagagggtgaagattaagagcatcgacgatgtcaagcaggtgctggacaaggatagcaacttcattattggaaaaatcacactcccctttaagaaggagtggcagaggctgtacagggagtggcaaaacaccacaatcaaggacgattacgagttcctgaagagcttctttaacgtgaagagcattacaaagctgcacaagaaggtcaggaaagacttcagcctccccattagcaccaacgagggaaagttcctggtgaagaggaagacctgggacaacaacttcatctaccagatcctcaatgactccgacagcagggccgacggcacaaagccctttatccctgccttcgacatcagcaagaacgaaatcgtggaggccatcatcgattcctttaccagcaaaaacattttctggctgcccaaaaatattgaactccagaaggtcgacaacaaaaacatctttgctatcgacacatccaaatggtttgaagtcgagacaccttccgacctgagggatatcggaattgccaccattcaatataagatcgacaataatagcaggcctaaagtgagggtcaaactcgactacgtgatcgacgacgacagcaagatcaactacttcatgaaccacagcctgctgaagtccaggtatcccgacaaggtcctcgaaatcctcaagcagagcaccatcattgaatttgagtccagcggattcaacaagacaatcaaagagatgctgggcatgaaactcgccggcatctataacgagaccagcaataac

SEQ ID NO: 10 - RNA, 63 nt, Homo sapiens
uaucaggcaguaccacaagcucguaauuaauaaaccaugaaaguaugguuuauuagauuguug

SEQ ID NO: 11 - RNA, 44 nt, Homo sapiens
cucguaauuaauaaaccaugaaaguaugguuuauuagauuguug

SEQ ID NO: 12 - RNA, 87 nt, Homo sapiens
guaucaggcaguaccacaagcucguaauuaauaaaccaugaaaguaugguuuauuagauuguugaaggcuaguccguuaucaacuug

SEQ ID NO: 13 - RNA, 46 nt, Artificial Sequence
  Synthetic Construct
  misc_feature (1)..(1): where n is any nucleotide
  misc_feature (46)..(46): where n is any nucleotide
ncucguaauuaauaaaccaugaaaguaugguuuauuagauuguugn

SEQ ID NO: 14 - RNA, 14 nt, Artificial Sequence
  synthetic construct
  misc_feature (14)..(14): where n is any nucleotide
  misc_feature (14)..(14): where n is any nucleotide
  misc_feature (14)..(14): where n is any nucleotide
guaccaaauaauun

SEQ ID NO: 15 - RNA, 16 nt, Artificial sequence
  FTN_1103
  Unsure (9)..(9)
  Unsure (9)..(13)
  misc_feature (9)..(13): n is a, c, g, or u
aaauaugannnnnggu

SEQ ID NO: 16 - RNA, 111 nt, Artificial sequence
  ScaRNA
  mutation (4)..(8)
  Unsure (22)..(47)
  misc_feature (22)..(47): n is a, c, g, or u
  mutation (48)..(54)
  Unsure (59)..(111)
  misc_feature (59)..(111): n is a, c, g, or u
guaccaaauaauuaaugcucunnnnnnnnnnnnnnnnnnnnnnnnnngaccucuguuunnnnnnnnnnnnnnnnnnnnnnnnnnnnnnnnnnnnnnnnnnnnnnnnnnnnn

SEQ ID NO: 17 - RNA, 20 nt, Artificial Sequence
  tracrRNA mutant
  misc_feature (1)..(2): tracrRNA mutant
  mutation (13)..(17)
guuguuagauuauuugguau

SEQ ID NO: 18 - protein, 36 aa, Streptococcus pyogenes
  1-1368 Arginine-Rich Motif
TAEATRLKRTARRRYTRRKNRICYLQEIFSNEMAKV

SEQ ID NO: 19 - protein, 36 aa, Listeria monocytogenes
  1-1334 Arginine-Rich Motif
TAADRRMNRTARRRIERRRNRISYLQEIFALEMANI

SEQ ID NO: 20 - protein, 36 aa, Lactobacillus salivarius
  1-1149 Arginine-Rich Motif
TAAERRGFRTQRRRLNRRKWRLKLLEEIFDPYMAEV

SEQ ID NO: 21 - protein, 36 aa, Neisseria meningitidis
  1-1082 Arginine-Rich Motif
LAMARRLARSVRRLTRRRAHRLLRARRLLKREGVLQ

SEQ ID NO: 22 - protein, 31 aa, Legionella pneumophilia
  1-1372 Arginine-Rich Motif
LSQAQRRATRHRVRNKKRNQFVKRVALQLFQ

SEQ ID NO: 23 - protein, 35 aa, Burkholderiales spp.
  1-1428 Arginine-Rich Motif
FSSKSRTAVRHRVRSYKGFDLRRRLLLLVAEYQLL

SEQ ID NO: 24 - protein, 36 aa, Campylobacter jejuni
  1-984 Arginine-Rich Motif
LALPRRLARSARKRLARRKARLNHLKHLIANEFKLN

SEQ ID NO: 25 - protein, 33 aa, Francisella novicida
  1-1629 Arginine-Rich Motif
LLMNNRTARRHQRRGIDRKQLVKRLFKLIWTEQ

SEQ ID NO: 26 - protein, 35 aa, Streptococcus pyogenes
  1-1368 RuvC-III Motif
VMGRHKPENIVIEMARENQTTQKGQKNSRERMKRI

SEQ ID NO: 27 - protein, 34 aa, Listeria monocytogenes
  1-1334 RuvC-III Motif
IMGYPPQTIVVEMARENQTTVKGKNNSRPRYKSL

SEQ ID NO: 28 - protein, 30 aa, Lactobacillus salivarius
  1-1149 RuvC-III Motif
AMKCEPTSIAIEFTREKRKSKLTNTRYKKI

SEQ ID NO: 29 - protein, 37 aa, Neisseria meningitidis
  1-1082 RuvC-III Motif
RYGSPARIHIETAREVGKSFKDRKEIEKRQEENRKDR

SEQ ID NO: 30 - protein, 40 aa, Legionella pneumophilia
  1-1372 RuvC-III Motif
RMMQRLAYEIAMAKWEQIKHIPDNSSLLIPIYLEQNRFEF

SEQ ID NO: 31 - protein, 42 aa, Burkholderiales spp.
  1-1428 RuvC-III Motif
KAIDRNSWEVAKRIAEEVKKSVDFTNGTVKIPVAIEANSFNF

SEQ ID NO: 32 - protein, 37 aa, Campylobacter jejuni
  1-984 RuvC-III Motif
KYGKVHKINIELAREVGKNHSQRAKIEKEQNENYKAK

SEQ ID NO: 33 - protein, 41 aa, Francisella novicida
  1-1629 RuvC-III Motif
KMATILAKNIVDDNWQNIKQVLSAKHQLHIPIITESNAFEF

SEQ ID NO: 34 - protein, 31 aa, Streptococcus pyogenes
  1-1368 RuvC-IV Motif
FYKVREINNYHHAHDAYLNAVVGTALIKKYP

SEQ ID NO: 35 - protein, 31 aa, Listeria monocytogenes
  1-1334 RuvC-IV Motif
LYKVREVNDYHHAHDAYLNGVVANTLLKVYP

SEQ ID NO: 36 - protein, 31 aa, Lactobacillus salivarius
  1-1149 RuvC-IV Motif
LIKNREVNDYHHAIDGYLTTFVGQYLYKVYP

SEQ ID NO: 37 - protein, 31 aa, Neisseria meningitidis
  1-1082 RuvC-IV Motif
LRKVRAENDRHHALDAVVVACSTVAMQQKIT

SEQ ID NO: 38 - protein, 31 aa, Legionella pneumophilia
  1-1372 RuvC-IV Motif
LVKSRQQSFPSHAIDATLTMSIGLKEFPQFS

SEQ ID NO: 39 - protein, 30 aa, Burkholderiales spp.
  1-1428 RuvC-IV  Motif
FRKPKVQPVASHSIDAMCIYLAACSDPFKT

SEQ ID NO: 40 - protein, 31 aa, Campylobacter jejuni
  1-984 RuvC-IV Motif
FSAKDRNNHLHHAIDAVIIAYANNSIVKAFS

SEQ ID NO: 41 - protein, 33 aa, Francisella novicida
  1-1629 RuvC-IV Motif
YAKGDKPQASYSHLIDAMLAFCIAADEHRNDGS

SEQ ID NO: 42 - RNA, 39 nt, HCV
  5' UTR
ugcgaaaggccuugugguacugccugauagggcgcuugc

SEQ ID NO: 43 - RNA, 87 nt, HCV; identical to SEQ ID NO: 12
  5' UTR rgRNA

SEQ ID NO: 44 - RNA, 40 nt, HCV
  3' UTR
uucuugguggcuccaucuuagcccuagucacggcuagcug

SEQ ID NO: 45 - DNA, 87 bp, HCV
  3' UTR rgRNA
gtgactagggctaagatggacucguaauuaauaaaccaugaaaguaugguuuauuagauuguugaaggcuaguccguuaucaacuug